European Patent Specification EP 4 007 777 B1, published October 11, 2023. Title: CAR T-cells for the treatment of Multiple myeloma. Applicant: Fundacio Clínic per  a la Recerca Biomedica Hospital Clínic de Barcelona Institut d’Investigacions Biomèdiques August Pi i Sunyer (IDIBAPS) Universitat de Barcelona. The sequence listing filed with the application follows.

SEQUENCE LISTING (16 sequences)

SEQ ID NO: 1 - protein, 120 aa, Artificial Sequence
  PEPTIDE 1..120
  VH domain
EVQLVESGGGLVQPGGSLRLSCAASGIDFSRYWMSWVRQAPGKGLEWIGEINPDSSTINYAPSLKDRFTISRDNAKNSLYLQMNSLRAEDTAVYYCASLYYDYGDAMDYWGQGTLVTVSS

SEQ ID NO: 2 - protein, 107 aa, Artificial Sequence
  PEPTIDE 1..107
  VL domain
DIQMTQSPSSLSASVGDRVTITCKASQSVDSNVAWYQQKPGKAPKALIFSASLRFSGVPSRFSGSGSGTDFTLTISSLQPEDFATYYCQQYNNYPLTFGGGTKVEIK

SEQ ID NO: 3 - protein, 242 aa, Artificial Sequence
  PEPTIDE 1..242
  VL and VH domain
EVQLVESGGGLVQPGGSLRLSCAASGIDFSRYWMSWVRQAPGKGLEWIGEINPDSSTINYAPSLKDRFTISRDNAKNSLYLQMNSLRAEDTAVYYCASLYYDYGDAMDYWGQGTLVTVSSGGGGSGGGGSGGGGSDIQMTQSPSSLSASVGDRVTITCKASQSVDSNVAWYQQKPGKAPKALIFSASLRFSGVPSRFSGSGSGTDFTLTISSLQPEDFATYYCQQYNNYPLTFGGGTKVEIK

SEQ ID NO: 4 - protein, 15 aa, Artificial Sequence
  PEPTIDE 1..15
  Linker
GGGGSGGGGSGGGGS

SEQ ID NO: 5 - protein, 20 aa, Artificial Sequence
  PEPTIDE 1..20
  signal peptide
MEAPAQLLFLLLLWLPDTTG

SEQ ID NO: 6 - protein, 262 aa, Artificial Sequence
  PEPTIDE 1..262
  BCMA -targeting moiety
MEAPAQLLFLLLLWLPDTTGEVQLVESGGGLVQPGGSLRLSCAASGIDFSRYWMSWVRQAPGKGLEWIGEINPDSSTINYAPSLKDRFTISRDNAKNSLYLQMNSLRAEDTAVYYCASLYYDYGDAMDYWGQGTLVTVSSGGGGSGGGGSGGGGSDIQMTQSPSSLSASVGDRVTITCKASQSVDSNVAWYQQKPGKAPKALIFSASLRFSGVPSRFSGSGSGTDFTLTISSLQPEDFATYYCQQYNNYPLTFGGGTKVEIK

SEQ ID NO: 7 - protein, 23 aa, Artificial Sequence
  PEPTIDE 1..23
  Transmembrane domain derived from CD8a
YIWAPLAGTCGVLLLSLVITLYC

SEQ ID NO: 8 - protein, 46 aa, Artificial Sequence
  PEPTIDE 1..46
  Hinge domain
TTTPAPRPPTPAPTIASQPLSLRPEACRPAAGGAVHTRGLDFACDI

SEQ ID NO: 9 - protein, 69 aa, Artificial Sequence
  PEPTIDE 1..69
  transmembrane domain further comprises a CD8 hinge
TTTPAPRPPTPAPTIASQPLSLRPEACRPAAGGAVHTRGLDFACDIYIWAPLAGTCGVLLLSLVITLYC

SEQ ID NO: 10 - protein, 113 aa, Artificial Sequence
  PEPTIDE 1..113
  Intracellular signaling domain
RVKFSRSADAPAYQQGQNQLYNELNLGRREEYDVLDKRRGRDPEMGGKPQRRKNPQEGLYNELQKDKMAEAYSEIGMKGERRRGKGHDGLYQGLSTATKDTYDALHMQALPPR

SEQ ID NO: 11 - protein, 42 aa, Artificial Sequence
  PEPTIDE 1..42
  costimulatory signaling domain
KRGRKKLLYIFKQPFMRPVQTTQEEDGCSCRFPEEEEGGCEL

SEQ ID NO: 12 - DNA, 1460 bp, Artificial Sequence
  full nucleotide sequence of the CAR
  misc_feature 1..1460
atggaggctccagcacagctcctttttctgctcctcctgtggctccctgatacgaccggagaagttcaactcgtggagagcggtgggggactcgtacagccaggtggatctctcagactttcctgcgctgcatcaggcatagactttagtcggtactggatgagttgggtacgacaagctcctgggaagggcttggaatggattggtgaaatcaacccggacagcagcaccataaattatgctccaagcttgaaagaccggttcactatatctcgggataatgctaaaaactccctttaccttcagatgaatagtctccgggcggaagatacggcggtgtattactgtgcttctctgtactacgactatggcgatgcaatggactattggggccaaggtacgctggtgaccgtctcatctggggggggaggtagtggaggaggaggttcaggggggggcggaagtgatattcaaatgacacagtctccgtcttcactgagtgcttctgtaggggatcgagttacgatcacttgtaaggccagccaatccgtggattctaatgttgcgtggtatcagcagaagcccggcaaagcgcctaaagcactgatatttagcgcatcactccgcttttccggggtcccctccaggttcagtggtagcgggtctggaacagacttcactctcactatatcttcattgcaaccagaagacttcgcgacctattactgtcagcaatacaataactacccgcttacgttcggcggcggcactaaagtcgaaatcaagacgacgacgccggcgccgagaccacctacacctgcaccaactattgcctctcagccactgagtctgcgccccgaggcatgtcgacctgccgctggcggggctgtgcacaccaggggcctagacttcgcctgcgatatctatatttgggctccactggcaggaacctgtggcgtgctgctgctgtctctggtcatcacactgtactgcaaaagaggcaggaagaaactgctgtatattttcaagcagccctttatgagacctgtgcagacaactcaggaggaagacgggtgcagctgtaggttccctgaggaagaggaaggaggctgtgagctgcgcgtgaaattttctcggagtgcagatgccccagcttaccagcagggccagaaccagctgtataacgagctgaatctggggcggagagaggaatacgacgtgctggataagaggcgcgggcgagatccagaaatgggaggaaaaccccagcgacggaagaaccctcaggagggactgtacaatgaactgcagaaggacaaaatggcagaggcctattccgaaatcgggatgaaaggagaaagaaggcgcggcaaggggcatgatggcctgtatcagggactgtcaaccgcaacaaaagatacttatgatgctctgcacatgcaggctctgcccccgcggta

SEQ ID NO: 13 - protein, 486 aa, Artificial Sequence
  PEPTIDE 1..486
  full amino acid sequence of the CAR
MEAPAQLLFLLLLWLPDTTGEVQLVESGGGLVQPGGSLRLSCAASGIDFSRYWMSWVRQAPGKGLEWIGEINPDSSTINYAPSLKDRFTISRDNAKNSLYLQMNSLRAEDTAVYYCASLYYDYGDAMDYWGQGTLVTVSSGGGGSGGGGSGGGGSDIQMTQSPSSLSASVGDRVTITCKASQSVDSNVAWYQQKPGKAPKALIFSASLRFSGVPSRFSGSGSGTDFTLTISSLQPEDFATYYCQQYNNYPLTFGGGTKVEIKTTTPAPRPPTPAPTIASQPLSLRPEACRPAAGGAVHTRGLDFACDIYIWAPLAGTCGVLLLSLVITLYCKRGRKKLLYIFKQPFMRPVQTTQEEDGCSCRFPEEEEGGCELRVKFSRSADAPAYQQGQNQLYNELNLGRREEYDVLDKRRGRDPEMGGKPQRRKNPQEGLYNELQKDKMAEAYSEIGMKGERRRGKGHDGLYQGLSTATKDTYDALHMQALPPR

SEQ ID NO: 14 - protein, 486 aa, Artificial Sequence
  MURINE (ARI2m)
MEAPAQLLFLLLLWLPDTTGQVQLQQSGGGLVQPGGSLKLSCAASGIDFSRYWMSWVRRAPGKGLEWIGEINPDSSTINYAPSLKDKFIISRDNAKNTLYLQMSKVRSEDTALYYCASLYYDYGDAMDYWGQGTSVTVSSGGGGSGGGGSGGGGSDIVMTQSQRFMTTSVGDRVSVTCKASQSVDSNVAWYQQKPRQSPKALIFSASLRFSGVPARFTGSGSGTDFTLTISNLQSEDLAEYFCQQYNNYPLTFGAGTKLELKTTTPAPRPPTPAPTIASQPLSLRPEACRPAAGGAVHTRGLDFACDIYIWAPLAGTCGVLLLSLVITLYCKRGRKKLLYIFKQPFMRPVQTTQEEDGCSCRFPEEEEGGCELRVKFSRSADAPAYQQGQNQLYNELNLGRREEYDVLDKRRGRDPEMGGKPQRRKNPQEGLYNELQKDKMAEAYSEIGMKGERRRGKGHDGLYQGLSTATKDTYDALHMQALPPR

SEQ ID NO: 15 - protein, 120 aa, Artificial Sequence
  murine VH
QVQLQQSGGGLVQPGGSLKLSCAASGIDFSRYWMSWVRRAPGKGLEWIGEINPDSSTINYAPSLKDKFIISRDNAKNTLYLQMSKVRSEDTALYYCASLYYDYGDAMDYWGQGTSVTVSS

SEQ ID NO: 16 - protein, 107 aa, Artificial Sequence
  Murine VL
DIVMTQSQRFMTTSVGDRVSVTCKASQSVDSNVAWYQQKPRQSPKALIFSASLRFSGVPARFTGSGSGTDFTLTISNLQSEDLAEYFCQQYNNYPLTFGAGTKLELK